European Patent Application EP 4 786 585 A1, published August 5, 2026. Title: Signal peptide for producing Serratia marcescens nuclease and use thereof. Applicant: CJ CheilJedang Corporation. Application KR. The sequence listing filed with the application follows.

SEQUENCE LISTING (16 sequences)

SEQ ID NO: 1 - protein, 245 aa, Serratia marcescens
DTLESIDNCAVGCPTGGSSNVSIVRHAYTLNNNSTTKFANWVAYHITKDTPASGKTRNWKTDPALNPADTLAPADYTGANAALKVDRGHQAPLASLAGVSDWESLNYLSNITPQKSDLNQGAWARLEDQERKLIDRADISSVYTVTGPLYERDMGKLPGTQKAHTIPSAYWKVIFINNSPAVNHYAAFLFDQNTPKGADFCQFRVTVDEIEKRTGLIIWAGLPDDVQASLKSKPGVLPELMGCKN

SEQ ID NO: 2 - DNA, 738 bp, Serratia marcescens
  source 1..738: mol_type = genomic DNA
gatacactggaatcaattgataattgcgcagttggctgcccgacgggcggcagctcaaatgtttcaattgtgagacacgcatacacattgaataataattcaacaacgaagtttgcaaattgggttgcatatcatattacaaaagatacaccggcaagcggcaaaacaagaaattggaaaacagatccggcactgaatccggcagatacactggcaccggcagattatacgggcgcaaatgcagcactgaaagttgatagaggccatcaagcaccgctggcatcactggcgggcgtttcagattgggaatcactgaattatctgtcaaatattacaccgcaaaaatcagatctgaatcaaggcgcatgggcaagactggaagatcaagaaagaaaactgattgatagagcagatatttcatcagtttatacagttacgggcccgctgtatgaaagagatatgggcaaactgccgggcacacaaaaagcacatacaattccgtcagcatattggaaagttatttttattaataattcaccggcagttaatcattatgcagcatttctgtttgatcaaaatacaccgaaaggcgcagatttttgccaatttagagttacagttgatgaaattgaaaaaagaacgggcctgattatttgggcgggcctgccggatgatgttcaagcatcactgaaatcaaaaccgggcgttctgccggaactgatgggctgcaaaaattga

SEQ ID NO: 3 - DNA, 43 bp, synthetic construct
  source 1..43: mol_type = other DNA
gcggccggtgcacatgatacactggaatcaattgataattgcg

SEQ ID NO: 4 - DNA, 41 bp, synthetic construct
  source 1..41: mol_type = other DNA
tgcaggtcgacaagctttcaatttttgcagcccatcagttc

SEQ ID NO: 5 - protein, 28 aa, synthetic construct
MFKKLLLATSALTFSLSLVLPLDGHAKA

SEQ ID NO: 6 - DNA, 84 bp, synthetic construct
  source 1..84: mol_type = other DNA
atgtttaagaaattacttttagcaacatctgcattaacattctctttatcattagttcttccgttggatggacatgccaaagct

SEQ ID NO: 7 - protein, 24 aa, synthetic construct
MKKMLMLAFTFLLALTIHVGEASA

SEQ ID NO: 8 - DNA, 72 bp, synthetic construct
  source 1..72: mol_type = other DNA
atgaaaaagatgttgatgttagcttttacatttcttttggctttgactatccatgtaggggaagcttcggct

SEQ ID NO: 9 - DNA, 39 bp, synthetic construct
  source 1..39: mol_type = other DNA
aggagagggacgcgtatgtttgcaaaacgattcaaaacc

SEQ ID NO: 10 - DNA, 33 bp, synthetic construct
  source 1..33: mol_type = other DNA
tgattccagtgtatcagcactcgcagccgccgg

SEQ ID NO: 11 - protein, 8 aa, synthetic construct
ETANKSNE

SEQ ID NO: 12 - DNA, 24 bp, synthetic construct
  source 1..24: mol_type = other DNA
gaaacggcgaacaaatcgaatgag

SEQ ID NO: 13 - DNA, 52 bp, synthetic construct
  source 1..52: mol_type = other DNA
gaaacggcgaacaaatcgaatgaggatacactggaatcaattgataattgcg

SEQ ID NO: 14 - DNA, 46 bp, synthetic construct
  source 1..46: mol_type = other DNA
ctcattcgatttgttcgccgtttcagctttggcatgtccatccaac

SEQ ID NO: 15 - DNA, 52 bp, synthetic construct; identical to SEQ ID NO: 13
  source 1..52: mol_type = other DNA

SEQ ID NO: 16 - DNA, 44 bp, synthetic construct
  source 1..44: mol_type = other DNA
ctcattcgatttgttcgccgtttcggccgaagcttcccctacat